European Patent Application EP 4 306 634 A1, published January 17, 2024. Title: Production method of low immunogenic retinal pigment epithelial cells. Applicant: RIKEN. The sequence listing filed with the application follows.

SEQUENCE LISTING (1 sequence)

SEQ ID NO: 1 - DNA, 23 bp, Homo sapiens
ataggaccagatgaagtgatcgg